European Patent Specification EP 3 763 819 B1, published November 19, 2025. Title: A novel promoter and preparation method of L-amino acid using thereof. Applicant: CJ CheilJedang Corporation. The sequence listing filed with the application follows.

SEQUENCE LISTING (9 sequences)

SEQ ID NO: 1 - DNA, 44 bp, Artificial Sequence
  LDH promoter region
tggtctgaccacattttcggacataatcgggcataagtaaaggt

SEQ ID NO: 2 - DNA, 44 bp, Corynebacterium glutamicum
tggtctgaccacattttcggacataatcgggcataattaaaggt

SEQ ID NO: 3 - DNA, 945 bp, Corynebacterium glutamicum
atgaaagaaaccgtcggtaacaagattgtcctcattggcgcaggcgatgtcggagttgcatacgcatatgcactgatcaaccaaggcatggcagaccaccttgcgatcatcgacattgatgaaaagaaactcgaaggcaacgtcaaggacttaaaccatggtgttgtgtgggccgattcccgcacccgcgtcactaagggaacctacgctgactgcgaagacgcagccatggttgtcatttgtgccggcgcagcccaaaagccaggcgagacccgcctccagctggtggacaaaaacgtcaagattatgaaatccatcgtcggcgatgtcatggacagcggattcgacggcatcttcctcgtggcgtccaacccagtggatatcctgacctacgcagtgtggaaattctccggcttggaatggaaccgcgtgatcggctccggaactgtcctggactccgctagattccgctacatgctcggcgaactctatgaagtggcaccaagctccgtccacgcctacatcatcggcgaacacggagacaccgaacttccagtcctgtcctccgcgaccatcgccggcgtatcgcttagccgaatgctggacaaagacccagagcttgagggccgtctagagaaaattttcgaagacacccgcgacgctgcctatcacattatcgacgccaagggctccacttcctacggcatcggcatgggtcttgctcgcatcacccgcgcaatcctacaaaaccaagacgttgcagtcccagtctctgcactgctccacggtgaatacggtgaggaagacatctacatcggcaccccagctgtggtgaaccgccgaggcatccgccgcgttgtcgaactagaaatcaccgaccacgagatggaacgcttcaagcattccgcaaataccctgcgcgaaattcagaagcagttcttctaa

SEQ ID NO: 4 - protein, 314 aa, Corynebacterium glutamicum
MKETVGNKIVLIGAGDVGVAYAYALINQGMADHLAIIDIDEKKLEGNVKDLNHGVVWADSRTRVTKGTYADCEDAAMVVICAGAAQKPGETRLQLVDKNVKIMKSIVGDVMDSGFDGIFLVASNPVDILTYAVWKFSGLEWNRVIGSGTVLDSARFRYMLGELYEVAPSSVHAYIIGEHGDTELPVLSSATIAGVSLSRMLDKDPELEGRLEKIFEDTRDAAYHIIDAKGSTSYGIGMGLARITRAILQNQDVAVPVSALLHGEYGEEDIYIGTPAVVNRRGIRRVVELEITDHEMERFKHSANTLREIQKQFF

SEQ ID NO: 5 - DNA, 75 bp, Artificial Sequence
  oligonucleotide
caagagcttgtgcccggattcctttgttacacctttacttatgcccgattatgtccgaaaatgtggtcagaccaa

SEQ ID NO: 6 - DNA, 32 bp, Artificial Sequence
  primer
cggtacccggggatcctgtgggtggcgttgta

SEQ ID NO: 7 - DNA, 33 bp, Artificial Sequence
  primer
ctttgttacacctttacttatgcccgattatgt

SEQ ID NO: 8 - DNA, 33 bp, Artificial Sequence
  primer
gtaaaggtgtaacaaaggaatccgggcacaagc

SEQ ID NO: 9 - DNA, 32 bp, Artificial Sequence
  primer
atgcctgcaggtcgacccacactgcgtaggtc